European Patent Specification EP 3 670 674 B1, published December 13, 2023. Title: COMPOSITIONS AND METHODS FOR DETECTING HUMAN PAPILLOMAVIRUS NUCLEIC ACID. Applicant: Gen-Probe Incorporated Schroder, Astrid. The sequence listing filed with the application follows.

SEQUENCE LISTING (161 sequences)

SEQ ID NO: 1 - DNA, 21 bp, Artificial Sequence
  Synthetic oligonucleotide
tcaagacactgaggaaaaacc

SEQ ID NO: 2 - DNA, 18 bp, Artificial Sequence
  synthetic oligonucleotide
gtttcaagacactgagga

SEQ ID NO: 3 - DNA, 21 bp, Artificial Sequence
  synthetic oligonucleotide
tatgtttcaagacactgagga

SEQ ID NO: 4 - DNA, 24 bp, Artificial Sequence
  synthetic oligonucleotide
acgactatgtttcaagacactgag

SEQ ID NO: 5 - DNA, 22 bp, Artificial Sequence
  synthetic oligonucleotide
gactatgtttcaagacactgag

SEQ ID NO: 6 - DNA, 20 bp, Artificial Sequence
  synthetic oligonucleotide
ctgcacgactatgtttcaag

SEQ ID NO: 7 - DNA, 24 bp, Artificial Sequence
  synthetic oligonucleotide
gtactgcacgactatgtttcaaga

SEQ ID NO: 8 - DNA, 19 bp, Artificial Sequence
  synthetic oligonucleotide
agtaaggtactgcacgact

SEQ ID NO: 9 - DNA, 19 bp, Artificial Sequence
  synthetic oligonucleotide
tagttgtctccaatgcttg

SEQ ID NO: 10 - DNA, 21 bp, Artificial Sequence
  synthetic oligonucleotide
atgttgtgtatagttgtctcc

SEQ ID NO: 11 - DNA, 24 bp, Artificial Sequence
  synthetic oligonucleotide
tagttcaatgttgtgtatagttgt

SEQ ID NO: 12 - DNA, 26 bp, Artificial Sequence
  Synthetic DNA and/or RNA oligonucleotide
ctgtagttcaatgttgtgtatagttg

SEQ ID NO: 13 - DNA, 21 bp, Artificial Sequence
  synthetic oligonucleotide
gcactgtagttcaatgttgtg

SEQ ID NO: 14 - DNA, 19 bp, Artificial Sequence
  synthetic oligonucleotide
cacgcactgtagttcaatg

SEQ ID NO: 15 - DNA, 21 bp, Artificial Sequence
  synthetic oligonucleotide
cattccacgcactgtagttca

SEQ ID NO: 16 - DNA, 23 bp, Artificial Sequence
  synthetic oligonucleotide
tgcattccacgcactgtagttca

SEQ ID NO: 17 - DNA, 46 bp, Artificial Sequence
  synthetic oligonucleotide
aatttaatacgactcactatagggagatagttgtctccaatgcttg

SEQ ID NO: 18 - DNA, 48 bp, Artificial Sequence
  synthetic oligonucleotide
aatttaatacgactcactatagggagaatgttgtgtatagttgtctcc

SEQ ID NO: 19 - DNA, 51 bp, Artificial Sequence
  synthetic oligonucleotide
aatttaatacgactcactatagggagatagttcaatgttgtgtatagttgt

SEQ ID NO: 20 - DNA, 53 bp, Artificial Sequence
  synthetic oligonucleotide
aatttaatacgactcactatagggagactgtagttcaatgttgtgtatagttg

SEQ ID NO: 21 - DNA, 48 bp, Artificial Sequence
  synthetic oligonucleotide
aatttaatacgactcactatagggagagcactgtagttcaatgttgtg

SEQ ID NO: 22 - DNA, 46 bp, Artificial Sequence
  synthetic oligonucleotide
aatttaatacgactcactatagggagacacgcactgtagttcaatg

SEQ ID NO: 23 - DNA, 48 bp, Artificial Sequence
  synthetic oligonucleotide
aatttaatacgactcactatagggagacattccacgcactgtagttca

SEQ ID NO: 24 - DNA, 50 bp, Artificial Sequence
  synthetic oligonucleotide
aatttaatacgactcactatagggagatgcattccacgcactgtagttca

SEQ ID NO: 25 - DNA, 20 bp, Artificial Sequence
  synthetic oligonucleotide
atgagcaattacccgacagc

SEQ ID NO: 26 - DNA, 18 bp, Artificial Sequence
  synthetic oligonucleotide
gagcaattacccgacagc

SEQ ID NO: 27 - DNA, 19 bp, Artificial Sequence
  synthetic oligonucleotide
tacccgacagctcagatga

SEQ ID NO: 28 - DNA, 20 bp, Artificial Sequence
  synthetic oligonucleotide
acccgacagctcagatgagg

SEQ ID NO: 29 - DNA, 22 bp, Artificial Sequence
  synthetic oligonucleotide
gacagctcagaggaggaggatg

SEQ ID NO: 30 - DNA, 20 bp, Artificial Sequence
  synthetic oligonucleotide
gctcagatgaggaggatgtc

SEQ ID NO: 31 - DNA, 20 bp, Artificial Sequence
  synthetic oligonucleotide
cagatgaggaggatgtcata

SEQ ID NO: 32 - DNA, 21 bp, Artificial Sequence
  synthetic oligonucleotide
atgaggaggatgtcatagaca

SEQ ID NO: 33 - DNA, 21 bp, Artificial Sequence
  synthetic oligonucleotide
aggaggatgtcatagacagtc

SEQ ID NO: 34 - DNA, 30 bp, Artificial Sequence
  synthetic oligonucleotide
cacacaaacgaagtgtagacttacactgac

SEQ ID NO: 35 - DNA, 22 bp, Artificial Sequence
  synthetic oligonucleotide
gtgtagacttacactgacaaca

SEQ ID NO: 36 - DNA, 23 bp, Artificial Sequence
  synthetic oligonucleotide
cgaagtgtagacttacactgaca

SEQ ID NO: 37 - DNA, 22 bp, Artificial Sequence
  synthetic oligonucleotide
caaacgaagtgtagacttacac

SEQ ID NO: 38 - DNA, 21 bp, Artificial Sequence
  synthetic oligonucleotide
cacacaaacgaagtgtagact

SEQ ID NO: 39 - DNA, 21 bp, Artificial Sequence
  synthetic oligonucleotide
ctctgtacacacaaacgaagt

SEQ ID NO: 40 - DNA, 22 bp, Artificial Sequence
  synthetic oligonucleotide
gtgtgctctgtacacacaaacg

SEQ ID NO: 41 - DNA, 22 bp, Artificial Sequence
  synthetic oligonucleotide
gaatatctacttgtgtgctctg

SEQ ID NO: 42 - DNA, 57 bp, Artificial Sequence
  synthetic oligonucleotide
aatttaatacgactcactatagggagacacacaaacgaagtgtagacttacactgac

SEQ ID NO: 43 - DNA, 49 bp, Artificial Sequence
  synthetic oligonucleotide
aatttaatacgactcactatagggagagtgtagacttacactgacaaca

SEQ ID NO: 44 - DNA, 50 bp, Artificial Sequence
  synthetic oligonucleotide
aatttaatacgactcactatagggagacgaagtgtagacttacactgaca

SEQ ID NO: 45 - DNA, 49 bp, Artificial Sequence
  synthetic oligonucleotide
aatttaatacgactcactatagggagacaaacgaagtgtagacttacac

SEQ ID NO: 46 - DNA, 48 bp, Artificial Sequence
  synthetic oligonucleotide
aatttaatacgactcactatagggagacacacaaacgaagtgtagact

SEQ ID NO: 47 - DNA, 48 bp, Artificial Sequence
  synthetic oligonucleotide
aatttaatacgactcactatagggagactctgtacacacaaacgaagt

SEQ ID NO: 48 - DNA, 49 bp, Artificial Sequence
  synthetic oligonucleotide
aatttaatacgactcactatagggagagtgtgctctgtacacacaaacg

SEQ ID NO: 49 - DNA, 49 bp, Artificial Sequence
  synthetic oligonucleotide
aatttaatacgactcactatagggagagaatatctacttgtgtgtgctc

SEQ ID NO: 50 - DNA, 24 bp, Artificial Sequence
  synthetic oligonucleotide
aaauguuugcuuuauauaugcacc

SEQ ID NO: 51 - DNA, 57 bp, Artificial Sequence
  synthetic oligonucleotide
aaauguuugcuuuauauaugcacctttaaaaaaaaaaaaaaaaaaaaaaaaaaaaaa

SEQ ID NO: 52 - DNA, 28 bp, Artificial Sequence
  synthetic oligonucleotide
gcucauaacaguggaggucaguugccuc

SEQ ID NO: 53 - DNA, 61 bp, Artificial Sequence
  synthetic oligonucleotide
gcucauaacaguggaggucaguugccuctttaaaaaaaaaaaaaaaaaaaaaaaaaaaaaa

SEQ ID NO: 54 - DNA, 20 bp, Artificial Sequence
  synthetic oligonucleotide
ccacgaacauugcaugauuu

SEQ ID NO: 55 - DNA, 23 bp, Artificial Sequence
  synthetic oligonucleotide
ccacgaacauugcaugauuugug

SEQ ID NO: 56 - DNA, 21 bp, Artificial Sequence
  synthetic oligonucleotide
cgaacauugcaugauuugugc

SEQ ID NO: 57 - DNA, 25 bp, Artificial Sequence
  synthetic oligonucleotide
ccacgaacauugcaugauuugugcc

SEQ ID NO: 58 - DNA, 22 bp, Artificial Sequence
  synthetic oligonucleotide
cgaacauugcaugauuugugcc

SEQ ID NO: 59 - DNA, 23 bp, Artificial Sequence
  synthetic oligonucleotide
cagcuggacaagcagaaccggac

SEQ ID NO: 60 - DNA, 22 bp, Artificial Sequence
  synthetic oligonucleotide
agcuggacaagcagaaccggac

SEQ ID NO: 61 - DNA, 23 bp, Artificial Sequence
  synthetic oligonucleotide
agcuggacaagcagaaccggaca

SEQ ID NO: 62 - DNA, 24 bp, Artificial Sequence
  synthetic oligonucleotide
cagcuggacaagcagaaccggaca

SEQ ID NO: 63 - DNA, 20 bp, Artificial Sequence
  synthetic oligonucleotide
cuggacaagcagaaccggac

SEQ ID NO: 64 - DNA, 25 bp, Artificial Sequence
  synthetic oligonucleotide
cuggacaagcagaaccggacacauc

SEQ ID NO: 65 - DNA, 26 bp, Artificial Sequence
  synthetic oligonucleotide
cuggacaagcagaaccggacacaucc

SEQ ID NO: 66 - DNA, 45 bp, Artificial Sequence
  synthetic oligonucleotide
agtaaggtactgcacgactatgtttcaagacactgaggaaaaacc

SEQ ID NO: 67 - DNA, 8 bp, Artificial Sequence
  Amp oligo core hybridizing sequence
gtttcaag

SEQ ID NO: 68 - DNA, 8 bp, Artificial Sequence
  Amp oligo core hybridizing sequence
acactgag

SEQ ID NO: 69 - DNA, 10 bp, Artificial Sequence
  synthetic oligonucleotide
ctgcacgact

SEQ ID NO: 70 - DNA, 52 bp, Artificial Sequence
  synthetic oligonucleotide
tgcattccacgcactgtagttcaatgttgtgtatagttgtctccaatgcttg

SEQ ID NO: 71 - DNA, 9 bp, Artificial Sequence
  Amp oligo core hybridizing sequence
ctgtagttc

SEQ ID NO: 72 - DNA, 8 bp, Artificial Sequence
  Amp oligo core hybridizing sequence
atgttgtg

SEQ ID NO: 73 - DNA, 10 bp, Artificial Sequence
  synthetic oligonucleotide
agttgtctcc

SEQ ID NO: 74 - DNA, 48 bp, Artificial Sequence
  synthetic oligonucleotide
atgagcaattacccgacagctcagakgaggaggatgtcatagacagtc

SEQ ID NO: 75 - DNA, 9 bp, Artificial Sequence
  Amp oligo core hybridizing sequence
aggaggatg

SEQ ID NO: 76 - DNA, 9 bp, Artificial Sequence
  Amp oligo core hybridizing sequence
cagakgagg

SEQ ID NO: 77 - DNA, 10 bp, Artificial Sequence
  synthetic oligonucleotide
acccgacagc

SEQ ID NO: 78 - DNA, 58 bp, Artificial Sequence
  synthetic oligonucleotide
gaatatctacttgtgtgctctgtacacacaaacgaagtgtagacttacactgacaaca

SEQ ID NO: 79 - DNA, 9 bp, Artificial Sequence
  Amp oligo core hybridizing sequence
gtgtagact

SEQ ID NO: 80 - DNA, 10 bp, Artificial Sequence
  synthetic oligonucleotide
cacacaaacg

SEQ ID NO: 81 - DNA, 9 bp, Artificial Sequence
  Amp oligo core hybridizing sequence
tgtgctctg

SEQ ID NO: 82 - DNA, 27 bp, Artificial Sequence
  synthetic oligonucleotide
aatttaatacgactcactatagggaga

SEQ ID NO: 83 - DNA, 866 bp, Human papillomavirus type 33
  ref <308>: M12732.1  GI:333049
  ref <309>: 1994-03-21
  ref <313>: (1)..(866)
gtaaactataatgccaagttttaaaaaagtagggtgtaaccgaaagcggttcaaccgaaaacggtgcatatataaagcaaacattttgcagtaaggtactgcacgactatgtttcaagacactgaggaaaaaccacgaacattgcatgatttgtgccaagcattggagacaactatacacaacattgaactacagtgcgtggaatgcaaaaaacctttgcaacgatctgaggtatatgattttgcatttgcagatttaacagttgtatatagagagggaaatccatttggaatatgtaaactgtgtttgcggttcttatctaaaattagtgaatatagacattataattattctgtatatggaaatacattagaacaaacagttaaaaaacctttaaatgaaatattaattaggtgtattatatgtcaaagacctttgtgtcctcaagaaaaaaaacgacatgtggatttaaacaaacgatttcataatatttcgggtcgttgggcagggcgctgtgcggcgtgttggaggtcccgacgtagagaaactgcactgtgacgtgtaaaaacgccatgagaggacacaagccaacgttaaaggaatatgttttagatttatatcctgaaccaactgacctatactgctatgagcaattaagtgacagctcagatgaggatgaaggcttggaccggccagatggacaagcacaaccagccacagctgattactacattgtaacctgttgtcacacttgtaacaccacagttcgtttatgtgtcaacagtacagcaagtgacctacgaaccatacagcaactacttatgggcacagtgaatattgtgtgccctacctgtgcacaacaataa

SEQ ID NO: 84 - DNA, 856 bp, Human papillomavirus type 31
  ref <308>: HQ537666.1  GI:337237882
  ref <309>: 2011-06-27
  ref <313>: (1)..(856)
taataataataatcttagtataaaaaagtagggagtgaccgaaagtggtgaaccgaaaacggttggtatataaagcacatagtattttgtgcaaacctacagacgccatgttcaaaaatcctgcagaaagacctcggaaattgcatgaactaagctcggcattggaaataccctacgatgaactaagattgaattgtgtctactgcaaaggtcagttaacagaaacagaggtattagattttgcatttacagatttaacaatagtatatagggacgacacaccacacggagtgtgtacaaaatgtttaagattttattcaaaagtaagtgaatttagatggtatagatatagtgtgtatggaacaacattagaaaaattgacaaacaaaggtatatgtgatttgttaattaggtgtataacgtgtcaaagaccgttgtgtccagaagaaaaacaaagacatttggataaaaagaaacgattccacaacataggaggaaggtggacaggacgttgcatagcatgttggagaagacctcgtactgaaacccaagtgtaaacatgcgtggagaaacacctacgttgcaagactatgtgttagatttgcaacctgaggcaactgacctccactgttatgagcaattacccgacagctcagatgaggaggatgtcatagacagtccagctggacaagcagaaccggacacatccaattacaatatcgttaccttttgttgtcagtgtaagtctacacttcgtttgtgtgtacagagcacacaagtagatattcgcatattgcaagagctgttaatgggctcatttggaatcgtgtgccccaactgttctactagactgtaa

SEQ ID NO: 85 - DNA, 22 bp, Artificial Sequence
  synthetic oligonucleotide
aggaggatgtcatagacaagtc

SEQ ID NO: 86 - DNA, 47 bp, Artificial Sequence
  synthetic oligonucleotide
aatttaatacgactcactatagggagagaatatctacttgtgtgctc

SEQ ID NO: 87 - DNA, 20 bp, Artificial Sequence
  synthetic oligonucleotide
gaatatctacttgtgtgctc

SEQ ID NO: 88 - DNA, 61 bp, Artificial Sequence
  synthetic oligonucleotide
gctcataacagtggaggtcagttgcctctttaaaaaaaaaaaaaaaaaaaaaaaaaaaaaa

SEQ ID NO: 89 - DNA, 58 bp, Artificial Sequence
  synthetic oligonucleotide
ctccaacacgctgcacagcgccctgtttaaaaaaaaaaaaaaaaaaaaaaaaaaaaaa

SEQ ID NO: 90 - DNA, 62 bp, Artificial Sequence
  synthetic oligonucleotide
gtgcacagatcaggtagcttgtagggtcgtttaaaaaaaaaaaaaaaaaaaaaaaaaaaaaa

SEQ ID NO: 91 - DNA, 61 bp, Artificial Sequence; identical to SEQ ID NO: 88
  synthetic oligonucleotide

SEQ ID NO: 92 - DNA, 28 bp, Artificial Sequence
  synthetic oligonucleotide
gctcataacagtggaggtcagttgcctc

SEQ ID NO: 93 - DNA, 62 bp, Artificial Sequence
  synthetic oligonucleotide
gugcacagaucagguagcuuguagggucgtttaaaaaaaaaaaaaaaaaaaaaaaaaaaaaa

SEQ ID NO: 94 - DNA, 29 bp, Artificial Sequence
  synthetic oligonucleotide
gugcacagaucagguagcuuguagggucg

SEQ ID NO: 95 - DNA, 25 bp, Artificial Sequence
  synthetic oligonucleotide
ctccaacacgctgcacagcgccctg

SEQ ID NO: 96 - DNA, 29 bp, Artificial Sequence
  synthetic oligonucleotide
gtgcacagatcaggtagcttgtagggtcg

SEQ ID NO: 97 - DNA, 28 bp, Artificial Sequence
  synthetic oligonucleotide
gctcataacagtggaggtcagttgcctc

SEQ ID NO: 98 - DNA, 40 bp, Artificial Sequence
  synthetic oligonucleotide
ttaartgacagctcagakgaggakgatgaaatagatggtc

SEQ ID NO: 99 - DNA, 14 bp, Artificial Sequence
  synthetic oligonucleotide
ctcagakgaggakg

SEQ ID NO: 100 - DNA, 21 bp, Artificial Sequence
  synthetic oligonucleotide
gtgacagctcagatgaggatg

SEQ ID NO: 101 - DNA, 22 bp, Artificial Sequence
  synthetic oligonucleotide
gacagctcagakgaggaggatg

SEQ ID NO: 102 - DNA, 27 bp, Artificial Sequence
  synthetic oligonucleotide
ctcagakgaggakgatgaaatagatgg

SEQ ID NO: 103 - DNA, 24 bp, Artificial Sequence
  synthetic oligonucleotide
rtgacagctcagakgaggakgatg

SEQ ID NO: 104 - DNA, 22 bp, Artificial Sequence
  synthetic oligonucleotide
gacagctcagatgaggaggatg

SEQ ID NO: 105 - DNA, 29 bp, Artificial Sequence
  synthetic oligonucleotide
tgacagctcagakgaggakgatgaaatag

SEQ ID NO: 106 - DNA, 50 bp, Artificial Sequence
  synthetic oligonucleotide
caatattgtaaccttttgttgcaagtgtgactctacgcttcggttgtgcg

SEQ ID NO: 107 - DNA, 13 bp, Artificial Sequence
  synthetic oligonucleotide
agagtcacacttg

SEQ ID NO: 108 - DNA, 46 bp, Artificial Sequence
  synthetic oligonucleotide
aatttaatacgactcactatagggagaacttgcaacaaaaggttac

SEQ ID NO: 109 - DNA, 55 bp, Artificial Sequence
  synthetic oligonucleotide
aatttaatacgactcactatagggagaacacttgcaacaaaaggttacaatattg

SEQ ID NO: 110 - DNA, 49 bp, Artificial Sequence
  synthetic oligonucleotide
aatttaatacgactcactatagggagaagagtcacacttgcaacaaaag

SEQ ID NO: 111 - DNA, 50 bp, Artificial Sequence
  synthetic oligonucleotide
aatttaatacgactcactatagggagaagagtcacacttgcaacaaaagg

SEQ ID NO: 112 - DNA, 48 bp, Artificial Sequence
  synthetic oligonucleotide
aatttaatacgactcactatagggagagcacaaccgaagcgtagagtc

SEQ ID NO: 113 - DNA, 57 bp, Artificial Sequence
  synthetic oligonucleotide
aatttaatacgactcactatagggagacgcacaaccgaagcgtagagtcacacttgc

SEQ ID NO: 114 - DNA, 47 bp, Artificial Sequence
  synthetic oligonucleotide
aatttaatacgactcactatagggagaaagcgtagagtcacacttgc

SEQ ID NO: 115 - DNA, 49 bp, Artificial Sequence
  synthetic oligonucleotide
aatttaatacgactcactatagggagagcaacaaaaggttacaatattg

SEQ ID NO: 116 - DNA, 47 bp, Artificial Sequence
  synthetic oligonucleotide
aatttaatacgactcactatagggagagaagcgtagagtcacacttg

SEQ ID NO: 117 - DNA, 14 bp, Artificial Sequence
  synthetic oligonucleotide
caacaaaaggttac

SEQ ID NO: 118 - DNA, 19 bp, Artificial Sequence
  synthetic oligonucleotide
acttgcaacaaaaggttac

SEQ ID NO: 119 - DNA, 28 bp, Artificial Sequence
  synthetic oligonucleotide
acacttgcaacaaaaggttacaatattg

SEQ ID NO: 120 - DNA, 22 bp, Artificial Sequence
  synthetic oligonucleotide
agagtcacacttgcaacaaaag

SEQ ID NO: 121 - DNA, 23 bp, Artificial Sequence
  synthetic oligonucleotide
agagtcacacttgcaacaaaagg

SEQ ID NO: 122 - DNA, 21 bp, Artificial Sequence
  synthetic oligonucleotide
gcacaaccgaagcgtagagtc

SEQ ID NO: 123 - DNA, 30 bp, Artificial Sequence
  synthetic oligonucleotide
cgcacaaccgaagcgtagagtcacacttgc

SEQ ID NO: 124 - DNA, 20 bp, Artificial Sequence
  synthetic oligonucleotide
aagcgtagagtcacacttgc

SEQ ID NO: 125 - DNA, 22 bp, Artificial Sequence
  synthetic oligonucleotide
gcaacaaaaggttacaatattg

SEQ ID NO: 126 - DNA, 20 bp, Artificial Sequence
  synthetic oligonucleotide
gaagcgtagagtcacacttg

SEQ ID NO: 127 - DNA, 23 bp, Artificial Sequence
  synthetic oligonucleotide
cagckggacaagcagaaccggac

SEQ ID NO: 128 - DNA, 16 bp, Artificial Sequence
  synthetic oligonucleotide
cgacgagccgaaccac

SEQ ID NO: 129 - DNA, 17 bp, Artificial Sequence
  synthetic oligonucleotide
cgacgagccgaaccaca

SEQ ID NO: 130 - DNA, 16 bp, Artificial Sequence
  synthetic oligonucleotide
gacgagccgaaccaca

SEQ ID NO: 131 - DNA, 18 bp, Artificial Sequence
  synthetic oligonucleotide
cgacgagccgaaccacaa

SEQ ID NO: 132 - DNA, 17 bp, Artificial Sequence
  synthetic oligonucleotide
gacgagccgaaccacaa

SEQ ID NO: 133 - DNA, 16 bp, Artificial Sequence
  synthetic oligonucleotide
acgagccgaaccacaa

SEQ ID NO: 134 - DNA, 46 bp, Artificial Sequence
  synthetic oligonucleotide
aatttaatacgactcactatagggagagttcagaaacagctgctgg

SEQ ID NO: 135 - DNA, 48 bp, Artificial Sequence
  synthetic oligonucleotide
aatttaatacgactcactatagggagagtgttcagaaacagctgctgg

SEQ ID NO: 136 - DNA, 50 bp, Artificial Sequence
  synthetic oligonucleotide
aatttaatacgactcactatagggagagggtgttcagaaacagctgctgg

SEQ ID NO: 137 - DNA, 46 bp, Artificial Sequence
  synthetic oligonucleotide
aatttaatacgactcactatagggagagggtgttcagaaacagctg

SEQ ID NO: 138 - DNA, 45 bp, Artificial Sequence
  synthetic oligonucleotide
aatttaatacgactcactatagggagaacacacaaaggacagggt

SEQ ID NO: 139 - DNA, 46 bp, Artificial Sequence
  synthetic oligonucleotide
aatttaatacgactcactatagggagagacacacaaaggacagggt

SEQ ID NO: 140 - DNA, 49 bp, Artificial Sequence
  synthetic oligonucleotide
aatttaatacgactcactatagggagagcacaccacggacacacaaagg

SEQ ID NO: 141 - DNA, 50 bp, Artificial Sequence
  synthetic oligonucleotide
aatttaatacgactcactatagggagacacaccacggacacacaaaggac

SEQ ID NO: 142 - DNA, 47 bp, Artificial Sequence
  synthetic oligonucleotide
aatttaatacgactcactatagggagacacaccacggacacacaaag

SEQ ID NO: 143 - DNA, 48 bp, Artificial Sequence
  synthetic oligonucleotide
ccagcagctgtttctgaacaccctgtcctttgtgtgtccgtggtgtgc

SEQ ID NO: 144 - DNA, 19 bp, Artificial Sequence
  synthetic oligonucleotide
gttcagaaacagctgctgg

SEQ ID NO: 145 - DNA, 21 bp, Artificial Sequence
  synthetic oligonucleotide
gtgttcagaaacagctgctgg

SEQ ID NO: 146 - DNA, 23 bp, Artificial Sequence
  synthetic oligonucleotide
gggtgttcagaaacagctgctgg

SEQ ID NO: 147 - DNA, 19 bp, Artificial Sequence
  synthetic oligonucleotide
gggtgttcagaaacagctg

SEQ ID NO: 148 - DNA, 18 bp, Artificial Sequence
  synthetic oligonucleotide
acacacaaaggacagggt

SEQ ID NO: 149 - DNA, 19 bp, Artificial Sequence
  synthetic oligonucleotide
gacacacaaaggacagggt

SEQ ID NO: 150 - DNA, 22 bp, Artificial Sequence
  synthetic oligonucleotide
gcacaccacggacacacaaagg

SEQ ID NO: 151 - DNA, 23 bp, Artificial Sequence
  synthetic oligonucleotide
cacaccacggacacacaaaggac

SEQ ID NO: 152 - DNA, 20 bp, Artificial Sequence
  synthetic oligonucleotide
cacaccacggacacacaaag

SEQ ID NO: 153 - DNA, 21 bp, Artificial Sequence
  synthetic oligonucleotide
gcagacgaccuucgagcauuc

SEQ ID NO: 154 - DNA, 18 bp, Artificial Sequence
  synthetic oligonucleotide
cgucugcugagcuuucua

SEQ ID NO: 155 - DNA, 25 bp, Artificial Sequence
  synthetic oligonucleotide
guaguagaaagcucagcagacgacc

SEQ ID NO: 156 - DNA, 13 bp, Artificial Sequence
  synthetic oligonucleotide
guagaaaccucgc

SEQ ID NO: 157 - DNA, 21 bp, Artificial Sequence
  synthetic oligonucleotide
  misc_feature (18)..(18): n is a or g or c or t/u, unknown, or other.
guagagagcucggcagangac

SEQ ID NO: 158 - DNA, 20 bp, Artificial Sequence
  synthetic oligonucleotide
gugugacggcagaauugagc

SEQ ID NO: 159 - DNA, 20 bp, Artificial Sequence
  synthetic oligonucleotide
uguguguguguuguaagugu

SEQ ID NO: 160 - DNA, 15 bp, Artificial Sequence
  synthetic oligonucleotide
ucuucugccgagcuc

SEQ ID NO: 161 - DNA, 21 bp, Artificial Sequence
  synthetic oligonucleotide
guagagagcucggcagaggac